European Patent Application EP 4 321 527 A1, published February 14, 2024. Title: CELL PENETRATING PEPTIDE VARIANTS AND USES THEROF. Applicant: STEM MEDITECH CO.Ltd. The sequence listing filed with the application follows.

SEQUENCE LISTING (40 sequences)

SEQ ID NO: 1 - protein, 14 aa, Artificial Sequence
  ZF1
XXXXGXLDXHAKEX

SEQ ID NO: 2 - protein, 19 aa, Artificial Sequence
  2XR, 2XD, 4XY, 4XR, 9XG, 9XE, 19XL or 9XW
GXRCXNCGXLDHHAKECKX

SEQ ID NO: 3 - protein, 19 aa, Artificial Sequence
  ZF1 derivative
GDRCYNCGGLDHHAKECKL

SEQ ID NO: 4 - protein, 14 aa, Artificial Sequence
  CPP region
RRPKGKSMQKRRSK

SEQ ID NO: 5 - protein, 9 aa, Artificial Sequence
  TAT
RKKRRQRRR

SEQ ID NO: 6 - protein, 9 aa, Artificial Sequence
  R9
RRRRRRRRR

SEQ ID NO: 7 - protein, 8 aa, Artificial Sequence
  ZF1 derivative
PPQPKKCH

SEQ ID NO: 8 - protein, 14 aa, Artificial Sequence
  ZF2
CHFCQSISHMVASC

SEQ ID NO: 9 - protein, 22 aa, Artificial Sequence
  ZF2 derivative
PPQPKKCHFCQSISHMVASCPL

SEQ ID NO: 10 - protein, 27 aa, Artificial Sequence
  ZF2 derivative2
PPQPKKCHFCQSISHMVASCPLKAQQK

SEQ ID NO: 11 - protein, 60 aa, Artificial Sequence
  LPX101
RRPKGKSMQKRRSKGDRCYNCGGLDHHAKECKLPPQPKKCHFCQSISHMVASCPLKAQQK

SEQ ID NO: 12 - protein, 58 aa, Artificial Sequence
  LPX102
GSERRPKGKSMQKRRSKGDRCYNCGGLDHHAKECKLPPQPKKCHFCQSISHMVASCPL

SEQ ID NO: 13 - protein, 36 aa, Artificial Sequence
  LPX103
GSERRPKGKSMQKRRSKGDRCYNCGGLDHHAKECKL

SEQ ID NO: 14 - protein, 42 aa, Artificial Sequence
  LPX104
ERRPKGKSMQKRRSKGDRCYNCGGLDHHAKECKLPPQPKKCH

SEQ ID NO: 15 - protein, 36 aa, Artificial Sequence
  TAT104
RKKRRQRRRGDRCYNCGGLDHHAKECKLPPQPKKCH

SEQ ID NO: 16 - protein, 36 aa, Artificial Sequence
  R9-104
RRRRRRRRRGDRCYNCGGLDHHAKECKLPPQPKKCH

SEQ ID NO: 17 - protein, 42 aa, Artificial Sequence
  HTAT-104
HHHHHHRKKRRQRRRGDRCYNCGGLDHHAKECKLPPQPKKCH

SEQ ID NO: 18 - protein, 42 aa, Artificial Sequence
  HR9-104
HHHHHHRRRRRRRRRGDRCYNCGGLDHHAKECKLPPQPKKCH

SEQ ID NO: 19 - protein, 39 aa, Artificial Sequence
  LPH-103
HHHHHHRRPKGKSMQKRRSKGDRCYNCGGLDHHAKECKL

SEQ ID NO: 20 - protein, 47 aa, Artificial Sequence
  H-104
HHHHHHRRPKGKSMQKRRSKGDRCYNCGGLDHHAKECKLPPQPKKCH

SEQ ID NO: 21 - protein, 47 aa, Artificial Sequence
  H-104-1
HHHHHHRRPKGKSMQKRRSKGDRCYRCGGLDHHAKECKLPPQPKKCH

SEQ ID NO: 22 - protein, 47 aa, Artificial Sequence
  H-104-2
HHHHHHRRPKGKSMQKRRSKGDRCRNCGGLDHHAKECKLPPQPKKCH

SEQ ID NO: 23 - protein, 47 aa, Artificial Sequence
  H-104-3
HHHHHHRRPKGKSMQKRRSKGDRCRRCGGLDHHAKECKLPPQPKKCH

SEQ ID NO: 24 - protein, 34 aa, Artificial Sequence
  103-A1
ERRPKGKSMQKRRSKGDRCYRCGGLDHHAKECKL

SEQ ID NO: 25 - protein, 34 aa, Artificial Sequence
  103-A2
ERRPKGKSMQKRRSKGDRCRNCGGLDHHAKECKL

SEQ ID NO: 26 - protein, 34 aa, Artificial Sequence
  103-A3
ERRPKGKSMQKRRSKGDRCRRCGGLDHHAKECKL

SEQ ID NO: 27 - protein, 34 aa, Artificial Sequence
  103-S1
ERRPKGKSMQKRRSKGRRCYNCGGLDHHAKECKL

SEQ ID NO: 28 - protein, 34 aa, Artificial Sequence
  LPS-103
ERRPKGKSMQKRRSKGDRCYNCGELDHHAKECKL

SEQ ID NO: 29 - protein, 34 aa, Artificial Sequence
  103-S1 #19
ERRPKGKSMQKRRSKGDRCYNCGGLDHHAKECKW

SEQ ID NO: 30 - protein, 34 aa, Artificial Sequence
  103-AS1
ERRPKGKSMQKRRSKGRRCRRCGGLDHHAKECKW

SEQ ID NO: 31 - protein, 34 aa, Artificial Sequence
  103-AS1 #21
ERRPKGKSMQKRRSKGRRCRRCGELDHHAKECKW

SEQ ID NO: 32 - protein, 36 aa, Artificial Sequence
  103-N1
GSERRPKGKSMQKRRSKGDRAYNCGGLDHHAKECKL

SEQ ID NO: 33 - protein, 36 aa, Artificial Sequence
  103-N2
GSERRPKGKSMQKRRSKGDRCYNAGGLDHHAKECKL

SEQ ID NO: 34 - protein, 36 aa, Artificial Sequence
  103-N3
GSERRPKGKSMQKRRSKGDRCYNCGGLDAHAKECKL

SEQ ID NO: 35 - protein, 36 aa, Artificial Sequence
  103-N4
GSERRPKGKSMQKRRSKGDRCYNCGGLDHHAKEAKL

SEQ ID NO: 36 - protein, 36 aa, Artificial Sequence
  103-N5
GSERRPKGKSMQKRRSKGDRCYDCGGLDHHAKECKL

SEQ ID NO: 37 - protein, 33 aa, Artificial Sequence
  LPX105
RRPKGKSMQKRRSKGDRCYNCGGLDHHAKECKL

SEQ ID NO: 38 - protein, 33 aa, Artificial Sequence
  LPS105
RRPKGKSMQKRRSKGDRCYNCGELDHHAKECKL

SEQ ID NO: 39 - protein, 39 aa, Artificial Sequence; identical to SEQ ID NO: 19
  LPH105

SEQ ID NO: 40 - protein, 39 aa, Artificial Sequence
  LPHS105
HHHHHHRRPKGKSMQKRRSKGDRCYNCGELDHHAKECKL